European Patent Application EP 4 400 094 A1, published July 17, 2024. Title: 거대 생리활성 물질 및 부형제를 포함하는 약학 조성물. Applicant: D&D Pharmatech. Application KR 10-2021-0118832, filed September 7, 2021. The sequence listing filed with the application follows.

SEQUENCE LISTING (17 sequences)

SEQ ID NO: 1 - protein, 39 aa, synthetic construct
HGEGTFTSDLSKQMEEEAVRLFIEWLKNGGPSSGAPPPS

SEQ ID NO: 2 - protein, 40 aa, synthetic construct
HGEGTFTSDLSKQMEEEAVRLFIEWLKNGGPSSGAPPPSC

SEQ ID NO: 3 - protein, 40 aa, synthetic construct
HGEGTFTSDLSKQMEEEAVRLFIEWLKNGGPSSGAPPPSK

SEQ ID NO: 4 - protein, 40 aa, synthetic construct
  SITE 2: note = X is 2-Aminoisobutyric acid(Aib); note (original language) = X는 2-아미노이소부티르산(Aib)
HXGEGTFTSDLSKQMEEEAVRLFIEWLKNGGPSSGAPPPS

SEQ ID NO: 5 - protein, 40 aa, synthetic construct
  SITE 2: note = X is 2-Aminoisobutyric acid(Aib); note (original language) = X는 2-아미노이소부티르산(Aib)
HXEGTFTSDLSKQMEEEAVRLFIEWLKNGGPSSGAPPPSK

SEQ ID NO: 6 - protein, 31 aa, synthetic construct
  SITE 2: note = X is 2-Aminoisobutyric acid(Aib); note (original language) = X는 2-아미노이소부티르산(Aib)
HXEGTFTSDVSSYLEGQAAKEFIAWLVRGRG

SEQ ID NO: 7 - protein, 30 aa, synthetic construct
  SITE 2: note = X is 2-Aminoisobutyric acid(Aib); note (original language) = X는 2-아미노이소부티르산(Aib)
HXQGTFTSDYSKYLDEQAAKEFVQWLMNTC

SEQ ID NO: 8 - protein, 30 aa, synthetic construct
  SITE 2: note = X is 2-Aminoisobutyric acid(Aib); note (original language) = X는 2-아미노이소부티르산(Aib)
HXQGTFTSDYSKYLDEQAAKEFVQWLMNTK

SEQ ID NO: 9 - protein, 40 aa, synthetic construct
  SITE 2: note = X is 2-Aminoisobutyric acid(Aib); note (original language) = X는 2-아미노이소부티르산(Aib)
YXQGTFTSDYSKLLDYMMQRDFVQWLLEGGPSSGAPPPSK

SEQ ID NO: 10 - protein, 21 aa, Homo sapiens
GIVEQCCTSICSLYQLENYCN

SEQ ID NO: 11 - protein, 30 aa, Homo sapiens
FVNQHLCGSHLVEALYLVCGERGFFYTPKT

SEQ ID NO: 12 - protein, 21 aa, synthetic construct
GIVEQCCTSICSLEQLENYCN

SEQ ID NO: 13 - protein, 34 aa, Homo sapiens
SVSEIQLMHNLGKHLNSMERVEWLRKKLQDVHNF

SEQ ID NO: 14 - protein, 37 aa, synthetic construct
KCNTATCATQRLANFLVHSSNNFGPILPPTNVGSNTY

SEQ ID NO: 15 - protein, 37 aa, synthetic construct
KCNTATCATQRLADFLRHSSPNFGAIPSSTNVGSRTY

SEQ ID NO: 16 - protein, 37 aa, synthetic construct
KCNTATCATQRLADFLRHSSNNFGAIPSSTNVGSRTY

SEQ ID NO: 17 - protein, 37 aa, synthetic construct
RCNTATCATQRLADFLRHSSNNFGAIPSSTNVGSKTY